European Patent Application EP 4 400 509 A1, published July 17, 2024. Title: Compound, compound salt, reagent for modification of antibody, production method for modified antibody and modified antibody. Applicant: Kagoshima University. Application WO. The sequence listing filed with the application follows.

SEQUENCE LISTING (155 sequences)

SEQ ID NO: 1 - protein, 13 aa, synthetic construct
  REGION 1..13: note = Fc binding peptide
  SITE 6: note = MISC_FEATURE - X is K, C, D, E, R, V, F, L, 2-Aminooctanedioic acid, Dpr, Orn,AcOrn, AcDab, Dab, Nle, Nva, Tle, Ala(t-Bu), or Cha
DCAYHXGELVWCT

SEQ ID NO: 2 - protein, 17 aa, synthetic construct
  REGION 1..17: note = IgG binding peptide
  SITE 8: note = MISC_FEATURE - X is K, C, D, E, R, V, F, L, 2-Aminooctanedioic acid, Dpr, Orn,AcOrn, AcDab, Dab, Nle, Nva, Tle, Ala(t-Bu), or Cha
GPDCAYHXGELVWCTFH

SEQ ID NO: 3 - protein, 13 aa, synthetic construct
  REGION 1..13: note = IgG binding peptide
  SITE 6: note = MISC_FEATURE - X is K, C, D, E, R, V, F, L, 2-Aminooctanedioic acid, Dpr, Orn,AcOrn, AcDab, Dab, Nle, Nva, Tle, Ala(t-Bu), or Cha
RCAYHXGELVWCS

SEQ ID NO: 4 - protein, 17 aa, synthetic construct
  REGION 1..17: note = IgG binding peptide
  SITE 8: note = MISC_FEATURE - X is K, C, D, E, R, V, F, L, 2-Aminooctanedioic acid, Dpr, Orn,AcOrn, AcDab, Dab, Nle, Nva, Tle, Ala(t-Bu), or Cha
GPRCAYHXGELVWCSFH

SEQ ID NO: 5 - protein, 17 aa, synthetic construct
  REGION 1..17: note = IgG binding peptide
  SITE 8: note = MISC_FEATURE - X is K, C, D, E, R, V, F, L, 2-Aminooctanedioic acid, Dpr, Orn,AcOrn, AcDab, Dab, Nle, Nva, Tle, Ala(t-Bu), or Cha
SPDCAYHXGELVWCTFH

SEQ ID NO: 6 - protein, 17 aa, synthetic construct
  REGION 1..17: note = IgG binding peptide
  SITE 8: note = MISC_FEATURE - X is K, C, D, E, R, V, F, L, 2-Aminooctanedioic acid, Dpr, Orn,AcOrn, AcDab, Dab, Nle, Nva, Tle, Ala(t-Bu), or Cha
GDDCAYHXGELVWCTFH

SEQ ID NO: 7 - protein, 17 aa, synthetic construct
  REGION 1..17: note = IgG binding peptide
  SITE 8: note = MISC_FEATURE - X is K, C, D, E, R, V, F, L, 2-Aminooctanedioic acid, Dpr, Orn,AcOrn, AcDab, Dab, Nle, Nva, Tle, Ala(t-Bu), or Cha
GPSCAYHXGELVWCTFH

SEQ ID NO: 8 - protein, 17 aa, synthetic construct
  REGION 1..17: note = IgG binding peptide
  SITE 8: note = MISC_FEATURE - X is K, C, D, E, R, V, F, L, 2-Aminooctanedioic acid, Dpr, Orn,AcOrn, AcDab, Dab, Nle, Nva, Tle, Ala(t-Bu), or Cha
GPDCAYHXGELVWCSFH

SEQ ID NO: 9 - protein, 17 aa, synthetic construct
  REGION 1..17: note = IgG binding peptide
  SITE 8: note = MISC_FEATURE - X is K, C, D, E, R, V, F, L, 2-Aminooctanedioic acid, Dpr, Orn,AcOrn, AcDab, Dab, Nle, Nva, Tle, Ala(t-Bu), or Cha
GPDCAYHXGELVWCTHH

SEQ ID NO: 10 - protein, 17 aa, synthetic construct
  REGION 1..17: note = IgG binding peptide
  SITE 8: note = MISC_FEATURE - X is K, C, D, E, R, V, F, L, 2-Aminooctanedioic acid, Dpr, Orn,AcOrn, AcDab, Dab, Nle, Nva, Tle, Ala(t-Bu), or Cha
GPDCAYHXGELVWCTFY

SEQ ID NO: 11 - protein, 17 aa, synthetic construct
  REGION 1..17: note = IgG binding peptide
  SITE 8: note = MISC_FEATURE - X is K,C, D, E, R, V, F, L, 2-Aminooctanedioic acid, Dpr, Orn,AcOrn, AcDab, Dab, Nle, Nva, Tle, Ala(t-Bu), or Cha
SPDCAYHXGELVWCTFY

SEQ ID NO: 12 - protein, 17 aa, synthetic construct
  REGION 1..17: note = IgG binding peptide
  SITE 8: note = MISC_FEATURE - X is K, C, D, E, R, V, F, L, 2-Aminooctanedioic acid, Dpr, Orn,AcOrn, AcDab, Dab, Nle, Nva, Tle, Ala(t-Bu), or Cha
SDDCAYHXGELVWCTFY

SEQ ID NO: 13 - protein, 17 aa, synthetic construct
  REGION 1..17: note = IgG binding peptide
  SITE 8: note = MISC_FEATURE - X is K, C, D, E, R, V, F, L, 2-Aminooctanedioic acid, Dpr, Orn,AcOrn, AcDab, Dab, Nle, Nva, Tle, Ala(t-Bu), or Cha
RGNCAYHXGQLVWCTYH

SEQ ID NO: 14 - protein, 17 aa, synthetic construct
  REGION 1..17: note = IgG binding peptide
  SITE 2: note = MISC_FEATURE - X is homocysteine
  SITE 8: note = MISC_FEATURE - X is K, C, D, E, R, V, F, L, 2-Aminooctanedioic acid, Dpr, Orn,AcOrn, AcDab, Dab, Nle, Nva, Tle, Ala(t-Bu), or Cha
  SITE 16: note = MISC_FEATURE - X is homocysteine
GXDCAYHXGELVWCTXH

SEQ ID NO: 15 - protein, 19 aa, synthetic construct
  REGION 1..19: note = IgG binding peptide
  SITE 10: note = MISC_FEATURE - X is K, C, D, E, R, V, F, L, 2-Aminooctanedioic acid, Dpr, Orn,AcOrn, AcDab, Dab, Nle, Nva, Tle, Ala(t-Bu), or Cha
RRGPDCAYHXGELVWCTFH

SEQ ID NO: 16 - protein, 13 aa, synthetic construct
  REGION 1..13: note = IgG binding peptide
  SITE 6: note = MISC_FEATURE - X is K, C, D, E, R, V, F, L, 2-Aminooctanedioic acid, Dpr, Orn,AcOrn, AcDab, Dab, Nle, Nva, Tle, Ala(t-Bu), or Cha
DCTYHXGNLVWCT

SEQ ID NO: 17 - protein, 13 aa, synthetic construct
  REGION 1..13: note = IgG binding peptide
  SITE 6: note = MISC_FEATURE - X is K, C, D, E, R, V, F, L, 2-Aminooctanedioic acid, Dpr, Orn,AcOrn, AcDab, Dab, Nle, Nva, Tle, Ala(t-Bu), or Cha
DCAYHXGNLVWCT

SEQ ID NO: 18 - protein, 13 aa, synthetic construct
  REGION 1..13: note = IgG binding peptide
  SITE 6: note = MISC_FEATURE - X is K, C, D, E, R, V, F, L, 2-Aminooctanedioic acid, Dpr, Orn,AcOrn, AcDab, Dab, Nle, Nva, Tle, Ala(t-Bu), or Cha
DCTYHXGELVWCT

SEQ ID NO: 19 - protein, 13 aa, synthetic construct
  REGION 1..13: note = IgG binding peptide
  SITE 6: note = MISC_FEATURE - X is K, C, D, E, R, V, F, L, 2-Aminooctanedioic acid, Dpr, Orn,AcOrn, AcDab, Dab, Nle, Nva, Tle, Ala(t-Bu), or Cha
DCAWHXGELVWCT

SEQ ID NO: 20 - protein, 13 aa, synthetic construct
  REGION 1..13: note = IgG binding peptide
  SITE 6: note = MISC_FEATURE - X is K, C, D, E, R, V, F, L, 2-Aminooctanedioic acid, Dpr, Orn,AcOrn, AcDab, Dab, Nle, Nva, Tle, Ala(t-Bu), or Cha
DCTYTXGNLVWCT

SEQ ID NO: 21 - protein, 13 aa, synthetic construct
  REGION 1..13: note = IgG binding peptide
  SITE 6: note = MISC_FEATURE - X is K, C, D, E, R, V, F, L, 2-Aminooctanedioic acid, Dpr, Orn,AcOrn, AcDab, Dab, Nle, Nva, Tle, Ala(t-Bu), or Cha
DCAYTXGNLVWCT

SEQ ID NO: 22 - protein, 13 aa, synthetic construct
  REGION 1..13: note = IgG binding peptide
  SITE 6: note = MISC_FEATURE - X is K, C, D, E, R, V, F, L, 2-Aminooctanedioic acid, Dpr, Orn,AcOrn, AcDab, Dab, Nle, Nva, Tle, Ala(t-Bu), or Cha
DCSYTXGNLVWCT

SEQ ID NO: 23 - protein, 13 aa, synthetic construct
  REGION 1..13: note = IgG binding peptide
  SITE 6: note = MISC_FEATURE - X is K, C, D, E, R, V, F, L, 2-Aminooctanedioic acid, Dpr, Orn,AcOrn, AcDab, Dab, Nle, Nva, Tle, Ala(t-Bu), or Cha
DCTWTXGNLVWCT

SEQ ID NO: 24 - protein, 13 aa, synthetic construct
  REGION 1..13: note = IgG binding peptide
  SITE 6: note = MISC_FEATURE - X is K, C, D, E, R, V, F, L, 2-Aminooctanedioic acid, Dpr, Orn,AcOrn, AcDab, Dab, Nle, Nva, Tle, Ala(t-Bu), or Cha
DCTYHXGNLVWCT

SEQ ID NO: 25 - protein, 13 aa, synthetic construct
  REGION 1..13: note = IgG binding peptide
  SITE 6: note = MISC_FEATURE - X is K, C, D, E, R, V, F, L, 2-Aminooctanedioic acid, Dpr, Orn,AcOrn, AcDab, Dab, Nle, Nva, Tle, Ala(t-Bu), or Cha
DCTYRXGNLVWCT

SEQ ID NO: 26 - protein, 13 aa, synthetic construct
  REGION 1..13: note = IgG binding peptide
  SITE 6: note = MISC_FEATURE - X is K, C, D, E, R, V, F, L, 2-Aminooctanedioic acid, Dpr, Orn,AcOrn, AcDab, Dab, Nle, Nva, Tle, Ala(t-Bu), or Cha
DCTYSXGNLVWCT

SEQ ID NO: 27 - protein, 13 aa, synthetic construct
  REGION 1..13: note = IgG binding peptide
  SITE 6: note = MISC_FEATURE - X is K, C, D, E, R, V, F, L, 2-Aminooctanedioic acid, Dpr, Orn,AcOrn, AcDab, Dab, Nle, Nva, Tle, Ala(t-Bu), or Cha
DCTYTXGNLVWCT

SEQ ID NO: 28 - protein, 13 aa, synthetic construct
  REGION 1..13: note = IgG binding peptide
  SITE 6: note = MISC_FEATURE - X is K, C, D, E, R, V, F, L, 2-Aminooctanedioic acid, Dpr, Orn,AcOrn, AcDab, Dab, Nle, Nva, Tle, Ala(t-Bu), or Cha
DCTYTXGELVWCT

SEQ ID NO: 29 - protein, 13 aa, synthetic construct
  REGION 1..13: note = IgG binding peptide
  SITE 6: note = MISC_FEATURE - X is K, C, D, E, R, V, F, L, 2-Aminooctanedioic acid, Dpr, Orn,AcOrn, AcDab, Dab, Nle, Nva, Tle, Ala(t-Bu), or Cha
DCTYTXGRLVWCT

SEQ ID NO: 30 - protein, 13 aa, synthetic construct
  REGION 1..13: note = IgG binding peptide
  SITE 6: note = MISC_FEATURE - X is K, C, D, E, R, V, F, L, 2-Aminooctanedioic acid, Dpr, Orn,AcOrn, AcDab, Dab, Nle, Nva, Tle, Ala(t-Bu), or Cha
DCTYTXGDLVWCT

SEQ ID NO: 31 - protein, 13 aa, synthetic construct
  REGION 1..13: note = IgG binding peptide
  SITE 6: note = MISC_FEATURE - X is K, C, D, E, R, V, F, L, 2-Aminooctanedioic acid, Dpr, Orn,AcOrn, AcDab, Dab, Nle, Nva, Tle, Ala(t-Bu), or Cha
DCTYTXGNLIWCT

SEQ ID NO: 32 - protein, 13 aa, synthetic construct
  REGION 1..13: note = IgG binding peptide
DCAYHRGELVWCT

SEQ ID NO: 33 - protein, 17 aa, synthetic construct
  REGION 1..17: note = IgG binding peptide
GPDCAYHRGELVWCTFH

SEQ ID NO: 34 - protein, 13 aa, synthetic construct
  REGION 1..13: note = IgG binding peptide
RCAYHRGELVWCS

SEQ ID NO: 35 - protein, 17 aa, synthetic construct
  REGION 1..17: note = IgG binding peptide
GPRCAYHRGELVWCSFH

SEQ ID NO: 36 - protein, 17 aa, synthetic construct
  REGION 1..17: note = IgG binding peptide
SPDCAYHRGELVWCTFH

SEQ ID NO: 37 - protein, 17 aa, synthetic construct
  REGION 1..17: note = IgG binding peptide
GDDCAYHRGELVWCTFH

SEQ ID NO: 38 - protein, 17 aa, synthetic construct
  REGION 1..17: note = IgG binding peptide
GPSCAYHRGELVWCTFH

SEQ ID NO: 39 - protein, 17 aa, synthetic construct
  REGION 1..17: note = IgG binding peptide
GPDCAYHRGELVWCSFH

SEQ ID NO: 40 - protein, 17 aa, synthetic construct
  REGION 1..17: note = IgG binding peptide
GPDCAYHRGELVWCTHH

SEQ ID NO: 41 - protein, 17 aa, synthetic construct
  REGION 1..17: note = IgG binding peptide
GPDCAYHRGELVWCTFY

SEQ ID NO: 42 - protein, 17 aa, synthetic construct
  REGION 1..17: note = IgG binding peptide
SPDCAYHRGELVWCTFY

SEQ ID NO: 43 - protein, 17 aa, synthetic construct
  REGION 1..17: note = IgG binding peptide
SDDCAYHRGELVWCTFY

SEQ ID NO: 44 - protein, 13 aa, synthetic construct
  REGION 1..13: note = IgG binding peptide
DCTYHRGNLVWCT

SEQ ID NO: 45 - protein, 13 aa, synthetic construct
  REGION 1..13: note = IgG binding peptide
DCAYHRGNLVWCT

SEQ ID NO: 46 - protein, 13 aa, synthetic construct
  REGION 1..13: note = IgG binding peptide
DCTYHRGELVWCT

SEQ ID NO: 47 - protein, 13 aa, synthetic construct
  REGION 1..13: note = IgG binding peptide
DCAWHRGELVWCT

SEQ ID NO: 48 - protein, 13 aa, synthetic construct
  REGION 1..13: note = IgG binding peptide
DCTYTNGNLVWCT

SEQ ID NO: 49 - protein, 13 aa, synthetic construct
  REGION 1..13: note = IgG binding peptide
DCAYTNGNLVWCT

SEQ ID NO: 50 - protein, 13 aa, synthetic construct
  REGION 1..13: note = IgG binding peptide
DCSYTNGNLVWCT

SEQ ID NO: 51 - protein, 13 aa, synthetic construct
  REGION 1..13: note = IgG binding peptide
DCTWTNGNLVWCT

SEQ ID NO: 52 - protein, 13 aa, synthetic construct
  REGION 1..13: note = IgG binding peptide
DCTYHNGNLVWCT

SEQ ID NO: 53 - protein, 13 aa, synthetic construct
  REGION 1..13: note = IgG binding peptide
DCTYRNGNLVWCT

SEQ ID NO: 54 - protein, 13 aa, synthetic construct
  REGION 1..13: note = IgG binding peptide
DCTYSNGNLVWCT

SEQ ID NO: 55 - protein, 13 aa, synthetic construct
  REGION 1..13: note = IgG binding peptide
DCTYTRGNLVWCT

SEQ ID NO: 56 - protein, 13 aa, synthetic construct
  REGION 1..13: note = IgG binding peptide
DCTYTNGELVWCT

SEQ ID NO: 57 - protein, 13 aa, synthetic construct
  REGION 1..13: note = IgG binding peptide
DCTYTNGRLVWCT

SEQ ID NO: 58 - protein, 13 aa, synthetic construct
  REGION 1..13: note = IgG binding peptide
DCTYTNGDLVWCT

SEQ ID NO: 59 - protein, 13 aa, synthetic construct
  REGION 1..13: note = IgG binding peptide
DCTYTNGNLIWCT

SEQ ID NO: 60 - protein, 22 aa, synthetic construct
  REGION 1..22: note = IgG binding peptide
GSGGSGPDCAYHRGELVWCTFH

SEQ ID NO: 61 - protein, 18 aa, synthetic construct
  REGION 1..18: note = IgG binding peptide
GSGGSDCAYHRGELVWCT

SEQ ID NO: 62 - protein, 23 aa, synthetic construct
  REGION 1..23: note = IgG binding peptide
KRRRGSGPDCAYHKGELVWCTFH

SEQ ID NO: 63 - protein, 23 aa, synthetic construct
  REGION 1..23: note = IgG binding peptide
KEEGGSGPDCAYHKGELVWCTFH

SEQ ID NO: 64 - protein, 17 aa, synthetic construct
  REGION 1..17: note = IgG binding peptide
GPDCAYHKGELVWCTFH

SEQ ID NO: 65 - protein, 22 aa, synthetic construct
  REGION 1..22: note = IgG binding peptide
RRRGSGPDCAYHKGELVWCTFH

SEQ ID NO: 66 - protein, 22 aa, synthetic construct
  REGION 1..22: note = IgG binding peptide
EEGGSGPDCAYHKGELVWCTFH

SEQ ID NO: 67 - protein, 19 aa, synthetic construct
  REGION 1..19: note = IgG binding peptide
KRRRGSDCAYHKGELVWCT

SEQ ID NO: 68 - protein, 19 aa, synthetic construct
  REGION 1..19: note = IgG binding peptide
KEEGGSDCAYHKGELVWCT

SEQ ID NO: 69 - protein, 13 aa, synthetic construct
  REGION 1..13: note = IgG binding peptide
DCAYHKGELVWCT

SEQ ID NO: 70 - protein, 18 aa, synthetic construct
  REGION 1..18: note = IgG binding peptide
RRRGSDCAYHKGELVWCT

SEQ ID NO: 71 - protein, 18 aa, synthetic construct
  REGION 1..18: note = IgG binding peptide
EEGGSDCAYHKGELVWCT

SEQ ID NO: 72 - protein, 34 aa, synthetic construct
  REGION 1..34: note = IgG binding peptide
FNMQCQRRFYEALHDPNLNEEQRNARIRSIRDDC

SEQ ID NO: 73 - protein, 35 aa, synthetic construct
  REGION 1..35: note = IgG binding peptide
GFNMQCQRRFYEALHDPNLNEEQRNARIRSIRDDC

SEQ ID NO: 74 - protein, 34 aa, synthetic construct
  REGION 1..34: note = IgG binding peptide
KNMQCQRRFYEALHDPNLNEEQRNARIRSIRDDC

SEQ ID NO: 75 - protein, 35 aa, synthetic construct
  REGION 1..35: note = IgG binding peptide
GFNMQCQKRFYEALHDPNLNEEQRNARIRSIRDDC

SEQ ID NO: 76 - protein, 34 aa, synthetic construct
  REGION 1..34: note = IgG binding peptide
KNMQCQKRFYEALHDPNLNEEQRNARIRSIRDDC

SEQ ID NO: 77 - protein, 33 aa, synthetic construct
  REGION 1..33: note = IgG binding peptide
FNMQQQRRFYEALHDPNLNEEQRNARIRSIRDD

SEQ ID NO: 78 - protein, 35 aa, synthetic construct
  REGION 1..35: note = IgG binding peptide
GKNMQCQRRFYEALHDPNLNEEQRNARIRSIRDDC

SEQ ID NO: 79 - protein, 40 aa, synthetic construct
  REGION 1..40: note = IgG binding peptide
FNMQQQRRFYEALHDPNLNEEQRNARIRSIRDDPSGSGSK

SEQ ID NO: 80 - protein, 40 aa, synthetic construct
  REGION 1..40: note = IgG binding peptide
FNMQCQRRFYEALHDPNLNEEQRNARIRSIRDDCSGSGSK

SEQ ID NO: 81 - protein, 34 aa, synthetic construct
  REGION 1..34: note = IgG binding peptide
FNMQQQRRFYEALHDPNLNEEQRNARIRSIRDDP

SEQ ID NO: 82 - protein, 33 aa, synthetic construct
  REGION 1..33: note = IgG binding peptide
FNMQQQCRFYEALHDPNLNEEQRNARIRSIRDD

SEQ ID NO: 83 - protein, 34 aa, synthetic construct
  REGION 1..34: note = IgG binding peptide
FNMQQQRRFYEALHDPNLNEEQRNARIRSIRDDC

SEQ ID NO: 84 - protein, 39 aa, synthetic construct
  REGION 1..39: note = IgG binding peptide
FNMQQQRRFYEALHDPNLNEEQRNARIRSIRDDPSRRKR

SEQ ID NO: 85 - protein, 39 aa, synthetic construct
  REGION 1..39: note = IgG binding peptide
FNMQQQRRFYEALHDPNLNEEQRNARIRSIRDDPSRRCR

SEQ ID NO: 86 - protein, 44 aa, synthetic construct
  REGION 1..44: note = IgG binding peptide
FNMQQQCRFYEALHDPNLNEEQRNARICSIRDDPSRRCRRCRRC

SEQ ID NO: 87 - protein, 44 aa, synthetic construct
  REGION 1..44: note = IgG binding peptide
FNMQQQKRFYEALHDPNLNEEQRNARIKSIRDDPSRRKRRKRRK

SEQ ID NO: 88 - protein, 33 aa, synthetic construct
  REGION 1..33: note = IgG binding peptide
KNMQQQCRFYEALHDPNLNEEQRNARIRSIRDD

SEQ ID NO: 89 - protein, 34 aa, synthetic construct
  REGION 1..34: note = IgG binding peptide
KNMQQQRRFYEALHDPNLNEEQRNARIRSIRDDC

SEQ ID NO: 90 - protein, 39 aa, synthetic construct
  REGION 1..39: note = IgG binding peptide
KNMQQQRRFYEALHDPNLNEEQRNARIRSIRDDPSRRKR

SEQ ID NO: 91 - protein, 39 aa, synthetic construct
  REGION 1..39: note = IgG binding peptide
KNMQQQRRFYEALHDPNLNEEQRNARIRSIRDDPSRRCR

SEQ ID NO: 92 - protein, 44 aa, synthetic construct
  REGION 1..44: note = IgG binding peptide
KNMQQQCRFYEALHDPNLNEEQRNARICSIRDDPSRRCRRCRRC

SEQ ID NO: 93 - protein, 44 aa, synthetic construct
  REGION 1..44: note = IgG binding peptide
KNMQQQKRFYEALHDPNLNEEQRNARIKSIRDDPSRRKRRKRRK

SEQ ID NO: 94 - protein, 34 aa, synthetic construct
  REGION 1..34: note = IgG binding peptide
GFNMQQQCRFYEALHDPNLNEEQRNARIRSIRDD

SEQ ID NO: 95 - protein, 35 aa, synthetic construct
  REGION 1..35: note = IgG binding peptide
GFNMQQQRRFYEALHDPNLNEEQRNARIRSIRDDC

SEQ ID NO: 96 - protein, 40 aa, synthetic construct
  REGION 1..40: note = IgG binding peptide
GFNMQQQRRFYEALHDPNLNEEQRNARIRSIRDDPSRRKR

SEQ ID NO: 97 - protein, 40 aa, synthetic construct
  REGION 1..40: note = IgG binding peptide
GFNMQQQRRFYEALHDPNLNEEQRNARIRSIRDDPSRRCR

SEQ ID NO: 98 - protein, 45 aa, synthetic construct
  REGION 1..45: note = IgG binding peptide
GFNMQQQCRFYEALHDPNLNEEQRNARICSIRDDPSRRCRRCRRC

SEQ ID NO: 99 - protein, 45 aa, synthetic construct
  REGION 1..45: note = IgG binding peptide
GFNMQQQKRFYEALHDPNLNEEQRNARIKSIRDDPSRRKRRKRRK

SEQ ID NO: 100 - protein, 34 aa, synthetic construct
  REGION 1..34: note = IgG binding peptide
FNMQCQZRFYEALHDPNLNEEQRNARIRSIRDDC

SEQ ID NO: 101 - protein, 34 aa, synthetic construct
  REGION 1..34: note = IgG binding peptide
KNMQCQZRFYEALHDPNLNEEQRNARIRSIRDDC

SEQ ID NO: 102 - protein, 40 aa, synthetic construct
  REGION 1..40: note = IgG binding peptide
GFNMQCQKRFYEALHDPNLNEEQRNARIRSIRDDCSRRKR

SEQ ID NO: 103 - protein, 34 aa, synthetic construct
  REGION 1..34: note = IgG binding peptide
FNMQCQKRFYEALHDPNLNEEQRNARIRSIRDDC

SEQ ID NO: 104 - protein, 39 aa, synthetic construct
  REGION 1..39: note = IgG binding peptide
KNMQCQKRFYEALHDPNLNEEQRNARIRSIRDDCSRRKR

SEQ ID NO: 105 - protein, 45 aa, synthetic construct
  REGION 1..45: note = IgG binding peptide
GFNMQCQKRFYEALHDPNLNEEQRNARIRSIRDDCSRRKRRKRRK

SEQ ID NO: 106 - protein, 44 aa, synthetic construct
  REGION 1..44: note = IgG binding peptide
KNMQCQKRFYEALHDPNLNEEQRNARIRSIRDDCSRRKRRKRRK

SEQ ID NO: 107 - protein, 45 aa, synthetic construct; identical to SEQ ID NO: 105
  REGION 1..45: note = IgG binding peptide

SEQ ID NO: 108 - protein, 11 aa, synthetic construct
  REGION 1..11: note = IgG binding peptide
CAWHLGELVWC

SEQ ID NO: 109 - protein, 13 aa, synthetic construct
  REGION 1..13: note = IgG binding peptide
DCAWHLGELVWCT

SEQ ID NO: 110 - protein, 13 aa, synthetic construct
  REGION 1..13: note = IgG binding peptide
DCAWHLGELVFCT

SEQ ID NO: 111 - protein, 13 aa, synthetic construct
  REGION 1..13: note = IgG binding peptide
  SITE 11: note = MISC_FEATURE - X is 1-naphtoyl, 2-naphtoyl, benzyl, or benzothiophene
DCAWHLGELVXCT

SEQ ID NO: 112 - protein, 15 aa, synthetic construct
  REGION 1..15: note = IgG binding peptide
CDCAWHLGELVWCTC

SEQ ID NO: 113 - protein, 11 aa, synthetic construct
  REGION 1..11: note = IgG binding peptide
CAYHLGELVWC

SEQ ID NO: 114 - protein, 14 aa, synthetic construct
  REGION 1..14: note = IgG binding peptide
DCAYHLGELVWCTF

SEQ ID NO: 115 - protein, 23 aa, synthetic construct
  REGION 1..23: note = IgG binding peptide
KRRRGSGPDCAYHKGELVWCTFH

SEQ ID NO: 116 - protein, 33 aa, synthetic construct
  REGION 1..33: note = IgG binding peptide
NMQCQRRFYEALHDPNLNEEQRNARIRSIRDDC

SEQ ID NO: 117 - protein, 34 aa, synthetic construct; identical to SEQ ID NO: 72
  REGION 1..34: note = IgG binding peptide

SEQ ID NO: 118 - protein, 33 aa, synthetic construct; identical to SEQ ID NO: 116
  REGION 1..33: note = IgG binding peptide

SEQ ID NO: 119 - protein, 34 aa, synthetic construct; identical to SEQ ID NO: 103
  REGION 1..34: note = IgG binding peptide

SEQ ID NO: 120 - protein, 33 aa, synthetic construct
  REGION 1..33: note = IgG binding peptide
NMQCQKRFYEALHDPNLNEEQRNARIRSIRDDC

SEQ ID NO: 121 - protein, 32 aa, synthetic construct
  REGION 1..32: note = IgG binding peptide
NMQQQRRFYEALHDPNLNEEQRNARIRSIRDD

SEQ ID NO: 122 - protein, 34 aa, synthetic construct; identical to SEQ ID NO: 74
  REGION 1..34: note = IgG binding peptide

SEQ ID NO: 123 - protein, 39 aa, synthetic construct
  REGION 1..39: note = IgG binding peptide
NMQQQRRFYEALHDPNLNEEQRNARIRSIRDDPSGSGSK

SEQ ID NO: 124 - protein, 39 aa, synthetic construct
  REGION 1..39: note = IgG binding peptide
NMQCQRRFYEALHDPNLNEEQRNARIRSIRDDCSGSGSK

SEQ ID NO: 125 - protein, 33 aa, synthetic construct
  REGION 1..33: note = IgG binding peptide
NMQQQRRFYEALHDPNLNEEQRNARIRSIRDDP

SEQ ID NO: 126 - protein, 32 aa, synthetic construct
  REGION 1..32: note = IgG binding peptide
NMQQQCRFYEALHDPNLNEEQRNARIRSIRDD

SEQ ID NO: 127 - protein, 33 aa, synthetic construct
  REGION 1..33: note = IgG binding peptide
NMQQQRRFYEALHDPNLNEEQRNARIRSIRDDC

SEQ ID NO: 128 - protein, 38 aa, synthetic construct
  REGION 1..38: note = IgG binding peptide
NMQQQRRFYEALHDPNLNEEQRNARIRSIRDDPSRRKR

SEQ ID NO: 129 - protein, 38 aa, synthetic construct
  REGION 1..38: note = IgG binding peptide
NMQQQRRFYEALHDPNLNEEQRNARIRSIRDDPSRRCR

SEQ ID NO: 130 - protein, 43 aa, synthetic construct
  REGION 1..43: note = IgG binding peptide
NMQQQCRFYEALHDPNLNEEQRNARICSIRDDPSRRCRRCRRC

SEQ ID NO: 131 - protein, 43 aa, synthetic construct
  REGION 1..43: note = IgG binding peptide
NMQQQKRFYEALHDPNLNEEQRNARIKSIRDDPSRRKRRKRRK

SEQ ID NO: 132 - protein, 32 aa, synthetic construct; identical to SEQ ID NO: 126
  REGION 1..32: note = IgG binding peptide

SEQ ID NO: 133 - protein, 33 aa, synthetic construct; identical to SEQ ID NO: 127
  REGION 1..33: note = IgG binding peptide

SEQ ID NO: 134 - protein, 38 aa, synthetic construct; identical to SEQ ID NO: 128
  REGION 1..38: note = IgG binding peptide

SEQ ID NO: 135 - protein, 38 aa, synthetic construct; identical to SEQ ID NO: 129
  REGION 1..38: note = IgG binding peptide

SEQ ID NO: 136 - protein, 43 aa, synthetic construct; identical to SEQ ID NO: 130
  REGION 1..43: note = IgG binding peptide

SEQ ID NO: 137 - protein, 43 aa, synthetic construct; identical to SEQ ID NO: 131
  REGION 1..43: note = IgG binding peptide

SEQ ID NO: 138 - protein, 33 aa, synthetic construct; identical to SEQ ID NO: 82
  REGION 1..33: note = IgG binding peptide

SEQ ID NO: 139 - protein, 34 aa, synthetic construct; identical to SEQ ID NO: 83
  REGION 1..34: note = IgG binding peptide

SEQ ID NO: 140 - protein, 39 aa, synthetic construct; identical to SEQ ID NO: 84
  REGION 1..39: note = IgG binding peptide

SEQ ID NO: 141 - protein, 39 aa, synthetic construct; identical to SEQ ID NO: 85
  REGION 1..39: note = IgG binding peptide

SEQ ID NO: 142 - protein, 44 aa, synthetic construct; identical to SEQ ID NO: 86
  REGION 1..44: note = IgG binding peptide

SEQ ID NO: 143 - protein, 44 aa, synthetic construct; identical to SEQ ID NO: 87
  REGION 1..44: note = IgG binding peptide

SEQ ID NO: 144 - protein, 33 aa, synthetic construct
  REGION 1..33: note = IgG binding peptide
NMQCQZRFYEALHDPNLNEEQRNARIRSIRDDC

SEQ ID NO: 145 - protein, 33 aa, synthetic construct; identical to SEQ ID NO: 144
  REGION 1..33: note = IgG binding peptide

SEQ ID NO: 146 - protein, 39 aa, synthetic construct
  REGION 1..39: note = IgG binding peptide
FNMQCQKRFYEALHDPNLNEEQRNARIRSIRDDCSRRKR

SEQ ID NO: 147 - protein, 33 aa, synthetic construct; identical to SEQ ID NO: 120
  REGION 1..33: note = IgG binding peptide

SEQ ID NO: 148 - protein, 38 aa, synthetic construct
  REGION 1..38: note = IgG binding peptide
NMQCQKRFYEALHDPNLNEEQRNARIRSIRDDCSRRKR

SEQ ID NO: 149 - protein, 44 aa, synthetic construct
  REGION 1..44: note = IgG binding peptide
FNMQCQKRFYEALHDPNLNEEQRNARIRSIRDDCSRRKRRKRRK

SEQ ID NO: 150 - protein, 43 aa, synthetic construct
  REGION 1..43: note = IgG binding peptide
NMQCQKRFYEALHDPNLNEEQRNARIRSIRDDCSRRKRRKRRK

SEQ ID NO: 151 - protein, 44 aa, synthetic construct; identical to SEQ ID NO: 149
  REGION 1..44: note = IgG binding peptide

SEQ ID NO: 152 - protein, 34 aa, synthetic construct; identical to SEQ ID NO: 72
  REGION 1..34: note = IgG binding peptide
  DISULFID 5..34: note = intrachain disulfide bond
  MOD_RES 1: note = hydrogen atom of amino group is replaced
  MOD_RES 34: note = carboxyl group is amidated

SEQ ID NO: 153 - protein, 33 aa, synthetic construct; identical to SEQ ID NO: 116
  REGION 1..33: note = IgG binding peptide
  DISULFID 4..33: note = intrachain disulfide bond
  MOD_RES 1: note = hydrogen atom of amino group is replaced
  MOD_RES 33: note = carboxyl group is amidated

SEQ ID NO: 154 - protein, 33 aa, synthetic construct
  REGION 1..33: note = a part of Trastuzumab
THTCPPCPAPELLGGPSVFLFPPKPKDTLMISR

SEQ ID NO: 155 - protein, 37 aa, synthetic construct
  REGION 1..37: note = a part of Trastuzumab
SCDKTHTCPPCPAPELLGGPSVFLFPPKPKDTLMISR